European Patent Specification EP 4 054 343 B1, published December 27, 2023. Title: Tolerogenic BLG peptides. Applicant: N.V. Nutricia. The sequence listing filed with the application follows.

SEQUENCE LISTING (74 sequences)

SEQ ID NO: 1 - protein, 48 aa, Artificial sequence
  AA 1-48
  misc_feature (1)..(1): Xaa can be Leu or Ile
XIVTQTMKGLDIQKVAGTWYSLAMAASDISLLDAQSAPLRVYVEELKP

SEQ ID NO: 2 - protein, 8 aa, Artificial sequence
  AA 13-20
QKVAGTWY

SEQ ID NO: 3 - protein, 8 aa, Artificial sequence
  AA 14-21
KVAGTWYS

SEQ ID NO: 4 - protein, 8 aa, Artificial sequence
  AA 15-22
VAGTWYSL

SEQ ID NO: 5 - protein, 8 aa, Artificial sequence
  AA 16-23
AGTWYSLA

SEQ ID NO: 6 - protein, 8 aa, Artificial sequence
  AA 17-24
GTWYSLAM

SEQ ID NO: 7 - protein, 8 aa, Artificial sequence
  AA 18-25
TWYSLAMA

SEQ ID NO: 8 - protein, 8 aa, Artificial sequence
  AA 19-26
WYSLAMAA

SEQ ID NO: 9 - protein, 8 aa, Artificial sequence
  AA 20-27
YSLAMAAS

SEQ ID NO: 10 - protein, 8 aa, Artificial sequence
  AA 21-28
SLAMAASD

SEQ ID NO: 11 - protein, 8 aa, Artificial sequence
  AA 22-29
LAMAASDI

SEQ ID NO: 12 - protein, 8 aa, Artificial sequence
  AA 23-30
AMAASDIS

SEQ ID NO: 13 - protein, 8 aa, Artificial sequence
  AA 24-31
MAASDISL

SEQ ID NO: 14 - protein, 8 aa, Artificial sequence
  AA 25-32
AASDISLL

SEQ ID NO: 15 - protein, 8 aa, Artificial sequence
  AA 26-33
ASDISLLD

SEQ ID NO: 16 - protein, 8 aa, Artificial sequence
  AA 27-34
SDISLLDA

SEQ ID NO: 17 - protein, 8 aa, Artificial sequence
  AA 28-35
DISLLDAQ

SEQ ID NO: 18 - protein, 8 aa, Artificial sequence
  AA 29-36
ISLLDAQS

SEQ ID NO: 19 - protein, 8 aa, Artificial sequence
  AA 30-37
SLLDAQSA

SEQ ID NO: 20 - protein, 8 aa, Artificial sequence
  AA 31-38
LLDAQSAP

SEQ ID NO: 21 - protein, 8 aa, Artificial sequence
  AA 32-39
LDAQSAPL

SEQ ID NO: 22 - protein, 8 aa, Artificial sequence
  AA 33-40
DAQSAPLR

SEQ ID NO: 23 - protein, 8 aa, Artificial sequence
  AA 34-41
AQSAPLRV

SEQ ID NO: 24 - protein, 8 aa, Artificial sequence
  AA 35-42
QSAPLRVY

SEQ ID NO: 25 - protein, 8 aa, Artificial sequence
  AA 36-43
SAPLRVYV

SEQ ID NO: 26 - protein, 8 aa, Artificial sequence
  AA 37-44
APLRVYVE

SEQ ID NO: 27 - protein, 8 aa, Artificial sequence
  AA 38-45
PLRVYVEE

SEQ ID NO: 28 - protein, 8 aa, Artificial sequence
  AA 39-46
LRVYVEEL

SEQ ID NO: 29 - protein, 8 aa, Artificial sequence
  AA 40-47
RVYVEELK

SEQ ID NO: 30 - protein, 8 aa, Artificial sequence
  AA 41-48
VYVEELKP

SEQ ID NO: 31 - protein, 10 aa, Artificial sequence
  AA 13-22
QKVAGTWYSL

SEQ ID NO: 32 - protein, 10 aa, Artificial sequence
  AA 14-23
KVAGTWYSLA

SEQ ID NO: 33 - protein, 10 aa, Artificial sequence
  AA 15-24
VAGTWYSLAM

SEQ ID NO: 34 - protein, 10 aa, Artificial sequence
  AA 16-25
AGTWYSLAMA

SEQ ID NO: 35 - protein, 10 aa, Artificial sequence
  AA 17-26
GTWYSLAMAA

SEQ ID NO: 36 - protein, 10 aa, Artificial sequence
  AA 18-27
TWYSLAMAAS

SEQ ID NO: 37 - protein, 10 aa, Artificial sequence
  AA 19-28
WYSLAMAASD

SEQ ID NO: 38 - protein, 10 aa, Artificial sequence
  AA 20-29
YSLAMAASDI

SEQ ID NO: 39 - protein, 10 aa, Artificial sequence
  AA 21-30
SLAMAASDIS

SEQ ID NO: 40 - protein, 10 aa, Artificial sequence
  AA 22-31
LAMAASDISL

SEQ ID NO: 41 - protein, 10 aa, Artificial sequence
  AA 23-32
AMAASDISLL

SEQ ID NO: 42 - protein, 10 aa, Artificial sequence
  AA 24-33
MAASDISLLD

SEQ ID NO: 43 - protein, 10 aa, Artificial sequence
  AA 25-34
AASDISLLDA

SEQ ID NO: 44 - protein, 10 aa, Artificial sequence
  AA 26-35
ASDISLLDAQ

SEQ ID NO: 45 - protein, 10 aa, Artificial sequence
  AA 27-36
SDISLLDAQS

SEQ ID NO: 46 - protein, 10 aa, Artificial sequence
  AA 28-37
DISLLDAQSA

SEQ ID NO: 47 - protein, 10 aa, Artificial sequence
  AA 29-38
ISLLDAQSAP

SEQ ID NO: 48 - protein, 10 aa, Artificial sequence
  AA 30-39
SLLDAQSAPL

SEQ ID NO: 49 - protein, 10 aa, Artificial sequence
  AA 31-40
LLDAQSAPLR

SEQ ID NO: 50 - protein, 10 aa, Artificial sequence
  AA 32-41
LDAQSAPLRV

SEQ ID NO: 51 - protein, 10 aa, Artificial sequence
  AA 33-42
DAQSAPLRVY

SEQ ID NO: 52 - protein, 10 aa, Artificial sequence
  AA 34-43
AQSAPLRVYV

SEQ ID NO: 53 - protein, 10 aa, Artificial sequence
  AA 35-44
QSAPLRVYVE

SEQ ID NO: 54 - protein, 10 aa, Artificial sequence
  AA 36-45
SAPLRVYVEE

SEQ ID NO: 55 - protein, 10 aa, Artificial sequence
  AA 37-46
APLRVYVEEL

SEQ ID NO: 56 - protein, 10 aa, Artificial sequence
  AA 38-47
PLRVYVEELK

SEQ ID NO: 57 - protein, 10 aa, Artificial sequence
  AA 39-48
LRVYVEELKP

SEQ ID NO: 58 - protein, 22 aa, Artificial sequence
  AA 1-22
  misc_feature (1)..(1): Xaa can be Leu or Ile
XIVTQTMKGLDIQKVAGTWYSL

SEQ ID NO: 59 - protein, 25 aa, Artificial sequence
  AA 1-25
  misc_feature (1)..(1): Xaa can be Leu or Ile
XIVTQTMKGLDIQKVAGTWYSLAMA

SEQ ID NO: 60 - protein, 26 aa, Artificial sequence
  AA 1-26
  misc_feature (1)..(1): Xaa can be Leu or Ile
XIVTQTMKGLDIQKVAGTWYSLAMAA

SEQ ID NO: 61 - protein, 30 aa, Artificial sequence
  AA 1-30
  misc_feature (1)..(1): Xaa can be Leu or Ile
XIVTQTMKGLDIQKVAGTWYSLAMAASDIS

SEQ ID NO: 62 - protein, 35 aa, Artificial sequence
  AA 1-35
  misc_feature (1)..(1): Xaa can be Leu or Ile
XIVTQTMKGLDIQKVAGTWYSLAMAASDISLLDAQ

SEQ ID NO: 63 - protein, 39 aa, Artificial sequence
  AA 1-39
  misc_feature (1)..(1): Xaa can be Leu or Ile
XIVTQTMKGLDIQKVAGTWYSLAMAASDISLLDAQSAPL

SEQ ID NO: 64 - protein, 42 aa, Artificial sequence
  AA 1-42
  misc_feature (1)..(1): Xaa can be Leu or Ile
XIVTQTMKGLDIQKVAGTWYSLAMAASDISLLDAQSAPLRVY

SEQ ID NO: 65 - protein, 31 aa, Artificial sequence
  AA 5-35
QTMKGLDIQKVAGTWYSLAMAASDISLLDAQ

SEQ ID NO: 66 - protein, 27 aa, Artificial sequence
  AA 1-27
  misc_feature (1)..(1): Xaa can be Leu or Ile
XIVTQTMKGLDIQKVAGTWYSLAMAAS

SEQ ID NO: 67 - protein, 32 aa, Artificial sequence
  AA 11-42
  misc_feature (1)..(1): Xaa can be Leu or Ile
DIQKVAGTWYSLAMAASDISLLDAQSAPLRVY

SEQ ID NO: 68 - protein, 30 aa, Artificial sequence
  AA 6-35
TMKGLDIQKVAGTWYSLAMAASDISLLDAQ

SEQ ID NO: 69 - protein, 27 aa, Artificial sequence
  AA 6-32
TMKGLDIQKVAGTWYSLAMAASDISLL

SEQ ID NO: 70 - protein, 32 aa, Artificial sequence
  AA 1-32
  misc_feature (1)..(1): Xaa can be Leu or Ile
XIVTQTMKGLDIQKVAGTWYSLAMAASDISLL

SEQ ID NO: 71 - protein, 18 aa, Artificial sequence
  AA 13-30
QKVAGTWYSLAMAASDIS

SEQ ID NO: 72 - protein, 18 aa, Artificial sequence
  AA-19-36
WYSLAMAASDISLLDAQS

SEQ ID NO: 73 - protein, 18 aa, Artificial sequence
  AA 25-42
AASDISLLDAQSAPLRVY

SEQ ID NO: 74 - protein, 18 aa, Artificial sequence
  AA 31-48
LLDAQSAPLRVYVEELKP